European Patent Application EP 4 667 580 A1, published December 24, 2025. Title: METHOD FOR SECRETORY PRODUCTION OF PROTEINS. Applicant: Ajinomoto Co., Inc. Application WO PCT/JP2024/005612, filed February 16, 2024. The sequence listing filed with the application follows.

SEQUENCE LISTING (48 sequences)

SEQ ID NO: 1 - DNA, 1458 bp, Corynebacterium glutamicum
  source 1..1458: mol_type = genomic DNA
atggaaaacccttatgtcgctgcgctcgatgacgataaaaaagaagtcggcgcaataaaagaagcagaaaaagaacctgaaataggtcccatcagagctgccggacgagccataccgctgcgcacccgcatcattttgatcgtggtgggtatcgccgggcttggtttgctggtcaacgcgattgctgtttccagcctcatgcgtgaagtttcctatacccgcatggatcaagagctagagacctcgatggggacgtgggcgcataacgttgagctgtttaatttcgatggcgtccgccaagggccacccagcgattattatgtggccaaggtttttcctgatggatccagcattattttcaacgatgcacaatcggcacccaatctagctgaaaccaccatcggtactggtccacacactgtggatgctgctagcggttctgcctccaacactccgtggcgtgtgatggcggaaaagaacggtgacattatcaccgtggtgggtaaaagcatggggcgtgaaacaaacctgctgtaccgattggtgatggtgcagatgatcatcggcgcgctgattctggttgctattttgattacttcactcttcctagtcagacgctcgttgcggccgttgagagaagttgaagagaccgccaccaggattgcgggcggtgatttggatcgacgtgtcccgcagtggccaatgaccacagaagtcggacagctgtcgaatgccctcaatatcatgttggagcagctccaagcctcaattctgaccgcccagcaaaaagaagctcagatgcgccgattcgttggcgacgcctcccacgagctccgcacaccactgacctctgtgaagggcttcaccgagctgtattcatcaggtgcaacagatgatgccaactgggtcatgtccaagatcggtggcgaagcccaacgcatgagtgtgcttgtggaagacctcctgtcactgacgcgtgccgaaggccagcaaatggagaagcaccgcgttgacgtgctggaactcgcattggcagtacgcggatccatgcgagcagcctggccagatcgcaccgtcaacgtgtccaataaagccgagtccattccagttgttgaaggcgacccaacccgcctccaccaagttctcaccaacctggttgccaacggactcaaccacggcggaccggacgcggaagtcagcattgagatcaacaccgatgggcaaaacgtgaggattctcgtggcagacaacggtgtcggaatgtctgaagaagatgcccagcatatcttcgagcgtttctaccgcgccgattcctcccgctcacgcgcatccggcggatcgggcctcggccttgcgatcacgaaatccctggtcgaaggccacggcggcacagtcaccgtcgacagcgtgcaaggcgaaggcacggtgttcacgatcaccttgccggcggtttcttaa

SEQ ID NO: 2 - protein, 485 aa, Corynebacterium glutamicum
MENPYVAALDDDKKEVGAIKEAEKEPEIGPIRAAGRAIPLRTRIILIVVGIAGLGLLVNAIAVSSLMREVSYTRMDQELETSMGTWAHNVELFNFDGVRQGPPSDYYVAKVFPDGSSIIFNDAQSAPNLAETTIGTGPHTVDAASGSASNTPWRVMAEKNGDIITVVGKSMGRETNLLYRLVMVQMIIGALILVAILITSLFLVRRSLRPLREVEETATRIAGGDLDRRVPQWPMTTEVGQLSNALNIMLEQLQASILTAQQKEAQMRRFVGDASHELRTPLTSVKGFTELYSSGATDDANWVMSKIGGEAQRMSVLVEDLLSLTRAEGQQMEKHRVDVLELALAVRGSMRAAWPDRTVNVSNKAESIPVVEGDPTRLHQVLTNLVANGLNHGGPDAEVSIEINTDGQNVRILVADNGVGMSEEDAQHIFERFYRADSSRSRASGGSGLGLAITKSLVEGHGGTVTVDSVQGEGTVFTITLPAVS

SEQ ID NO: 3 - protein, 485 aa, Corynebacterium glutamicum
MENPYVAALDDENQEVGVKKEAEKEPEIGPIRAAGRAIPLRTRIILIVVGIAGLGLLVNAIAVSSLMREVSYTRMDQELETSMGTWAHNVELFNFDGVRQGPPSDYYVAKVFPDGSSIIFNDAQSAPDLAETTIGTGPHTVDAASGSASNTPWRVMAEKNGDIITVVGKSMGRETNLLYRLVMVQMIIGALILVAILITSLFLVRRSLRPLREVEETATRIAGGDLDRRVPQWPMTTEVGQLSNALNIMLEQLQASILTAQQKEAQMRRFVGDASHELRTPLTSVKGFTELYSSGATDDANWVMSKIGGEAQRMSVLVEDLLSLTRAEGQQMEKHRVDVLELALAVRGSMRAAWPDRTVNVSNKAESIPVVKGDPTRLHQVLTNLVANGLNHGGPDAEVSIEINTDGQNVRILVADNGVGMSEEDAQHIFERFYRADSSRSRASGGSGLGLAITKSLVEGHGGTVTVDSVQGEGTVFTITLPAVS

SEQ ID NO: 4 - protein, 485 aa, Corynebacterium glutamicum
MENPYVAALDDENQEVGVKKEAEKEPEIGPIRAAGRAIPLRTRIILIVVGIAGLGLLVNAIAVSSLMREVSYTRMDQELETSMGTWAHNVELFNFDGVRQGPPSDYYVAKVFPDGSSIIFNDAQSAPDLAETTIGTGPHTVDAASGSASNTPWRVMAEKNGDIITVVGKSMGRETNLLYRLVVVQMIIGALILVAILITSLFLVRRSLRPLREVEETATRIAGGDLDRRVPQWPMTTEVGQLSNALNIMLEQLQASILTAQQKEAQMRRFVGDASHELRTPLTSVKGFTELYSSGATDDANWVMSKIGGEAQRMSVLVEDLLSLTRAEGQQMEKHRVDVLELALAVRGSMRAAWPDRTVNVSNKAESIPVVEGDPTRLHQVLTNLVANGLNHGGPDAEVSIEINTDGQNVRILVADNGVGMSEEDAQHIFERFYRADSSRSRASGGSGLGLAITKSLVEGHGGTVTVDSVQGEGTVFTITLPAVS

SEQ ID NO: 5 - protein, 504 aa, Corynebacterium callunae
MENPYVAALDKNSNFGAKDTDSAVSDSTEVSQNNDGIGTPATAEPKVGPIRTAGRAMPLRTRIILLVVGIAGLGLLVNAVAVSSLMREVSYTRMDQDLESAMGTWVRNVELFNFDGVRQGPPSDYYVAKVFPDGSSIIFNDAESAPDLGQTTIGTGPHTVEAAEGSASSTHWRVMAAKNGDVITVVGKSMGRESTLLYRLVVVQMVIGVLILIAILIGSFFLVRRSLKPLREVEETASRIAGGELDRRVPQWPMTTEVGQLANALNIMLEQLQTSIMNAQQKEAQMRRFVGDASHELRTPLTSVKGFTELYSSGATQDADWVLSKIGGEAQRMSVLVEDLLSLTRAEGQQMEKHRVDMLELALAVRGSLKAAWPDRTVNVANRSENIPVVEGDPTRLHQVLTNLVANGLNHGGPEAEVNIQVETADDKVKILVIDNGVGMSKEDAEHIFERFYRADTSRSRASGGSGLGLAITKSLVEGHGGTITVDSELGKGTVFSIILPAAE

SEQ ID NO: 6 - protein, 458 aa, Corynebacterium crenatum
IGPIRAAGRAIPLRTRIILIVVGIAGLGLLVNAIAVSSLMREVSYTRMDQELETSMGTWAHNVELFNFDGVRQGPPSDYYVAKVFPDGSSIIFNDAQSAPDLAETTIGTGPHTVDAASGSASNTPWRVMAEKNGDIITVVGKSMGRETNLLYRLVMVQMIIGALILVAILITSLFLVRRSLRPLREVEETATRIAGGDLDRRVPQWPMTTEVGQLSNALNIMLEQLQASILSAQQKEAQMRRFVGDASHELRTPLTSVKGFTELYSSGATDDANWVMSKIGGEAQRMSVLVEDLLSLTRAEGQQMEKHRVDVLELALAVRGSMRAAWPDRTVNVSNKAASIPVVEGDPTRLHQVLTNLVANGLNHGGPDAEVSIEINTDGQNVRILVADNGVGMSEEDAQHIFERFYRADSSRSRASGGSGLGLAITKSLVEGHGGTVTVDSVQGEGTVFTITLPAVS

SEQ ID NO: 7 - protein, 471 aa, Corynebacterium efficiens
MTAPENPHAQVTPVGRFRQAARGVPLRTRIILLVVGIAGLGLLVNAIAVSSLMREVSYSRMDQELESAMNSWAQTAELFGSITLGPPSDYYVVRIFPDGSHMVFNQSDSAPDLGETTIGIGPHTASAAPGSSSSVPWRVIAISDNGTITVVGKSLAPESMLLYRLVIVQLVIGMLIVVAILLSSLYLVNRSLRPLREVEKTAKSIAGGDLDRRVPQWPMTTEVGQLANALNIMLEQLQASILSAQEKESQMRRFVGDASHELRTPLTSVKGYSELYHSGATRDADWVLSKISGEAQRMSVLVEDLLSLTRAEGQQMEKRPVDVLELSLSVASSMRAAWPERSITVVNKTGSLPVVEGDATRLHQVLTNLVNNGLNHGGPDASVEIEISAEGGSVLVRVVDDGVGMTAEDAQHIFERFYRTDTSRSRASGGSGLGLAITKSLVEGHRGTITVDSEVGEGTVFTITLPSRMED

SEQ ID NO: 8 - DNA, 708 bp, Corynebacterium glutamicum
  source 1..708: mol_type = genomic DNA
atggacaaccagtctgacggacaaatccgcgtactcgtcgttgatgacgagccaaacatcgtcgagctgctcaccgtaagccttaaattccaaggcttcgcagtgatgaccgccaacgatggcaatgaagccctgaagattgctcgtgagttccgtccagacgcatacatcctcgatgtcatgatgccaggaatggacggcttcgagctgctgaccaagctgcgcggcgaaggccttgacagcccagttctgtacctcaccgcaaaggatgccgtggagcaccgcatccacggcctgaccatcggcgctgacgactacgtgaccaagcctttctccctggaagaagtaatcacccgcctgcgcgtgattcttcgtcgcggtggagcagttgaagaagacacctcaacttccctgcagtacgcagacctcaccctcaacgatgaaacccacgaggtcaccaaggctggcgaactgatcgatctttccccaactgaattcaacctcctgcgctacctcatgctcaacgctgaagtggtgctgtccaaggcaaagatcctggataacgtgtggcactacgattttggtggcgacggcaacgtcgtggaatcctacatctcctacctgcgccgcaaggtggacacccaggatccgcagctaattcagactgttcgtggcgttggatatgttctgcgcaccccacgtagctaa

SEQ ID NO: 9 - protein, 235 aa, Corynebacterium glutamicum
MDNQSDGQIRVLVVDDEPNIVELLTVSLKFQGFAVMTANDGNEALKIAREFRPDAYILDVMMPGMDGFELLTKLRGEGLDSPVLYLTAKDAVEHRIHGLTIGADDYVTKPFSLEEVITRLRVILRRGGAVEEDTSTSLQYADLTLNDETHEVTKAGELIDLSPTEFNLLRYLMLNAEVVLSKAKILDNVWHYDFGGDGNVVESYISYLRRKVDTQDPQLIQTVRGVGYVLRTPRS

SEQ ID NO: 10 - DNA, 1500 bp, Corynebacterium glutamicum
  source 1..1500: mol_type = genomic DNA
atgtttaacaaccgtatccgcactgcagctctcgctggtgcaatcgcaatctccaccgcagcttccggcgtagctatcccagcattcgctcaggagaccaacccaaccttcaacatcaacaacggcttcaacgatgctgatggatccaccatccagccagttgagccagttaaccacaccgaggaaaccctccgcgacctgactgactccaccggcgcttacctggaagagttccagtacggcaacgttgaggaaatcgttgaagcatacctgcaggttcaggcttccgcagacggattcgatccttctgagcaggctgcttacgaggctttcgaggctgctcgcgttcgtgcatcccaggagctcgcggcttccgctgagaccatcactaagacccgcgagtccgttgcttacgcactcaaggctgaccgcgaagctaccgcagctttcgaggcttacctcagcgctcttcgtcaggtttcagtcatcaacgatctgatcgctgatgctaacgccaagaacaagactgactttgcagagatcgagctctacgatgttctttacaccgacgccgacatctctggcgatgctccacttcttgctcctgcatacaaggagctgaaggaccttcaggctgaggttgacgcagacttcgagtggttgggcgagttcgcaattgataacaatgaagacaactacgtcattcgtactcacatccctgctgtagaggcactcaaggcagcgatcgattcactggtcgacaccgttgagccacttcgtgcagacgctatcgctaagaacatcgaggctcagaagtctgacgttctggttccccagctcttcctcgagcgtgcaactgcacagcgcgacaccctgcgtgttgtagaggcaatcttctctacctctgctcgttacgttgaactctacgagaacgtcgagaacgttaacgttgagaacaagacccttcgccagcactactcttccctgatccctaacctcttcatcgcagcggttggcaacatcaacgagctcaacaatgcagatcaggctgcacgtgagctcttcctcgattgggacaccgacctcaccaccaacgatgaggacgaagcttactaccaggctaagctcgacttcgctatcgagacctacgcaaagatcctgatcaacggtgaagtttggcaggagccactcgcttacgtccagaacctggatgcaggcgcacgtcaggaagcagctgaccgcgaagcagagcgcgcagctgacgcagcataccgcgctgagcagctccgcatcgctcaggaagcagctgacgctcagaaggctctcgctgaggctcttgctaatgcaggcaacaacgacaacggtggcgacaactcctccgacgacaagggaaccggttcttccgacatcggaacctggggacctttcgcagcaattgcagctatcatcgcagcaatcgcagctatcttcccattcctctccggtatcgttaagttctaa

SEQ ID NO: 11 - protein, 499 aa, Corynebacterium glutamicum
MFNNRIRTAALAGAIAISTAASGVAIPAFAQETNPTFNINNGFNDADGSTIQPVEPVNHTEETLRDLTDSTGAYLEEFQYGNVEEIVEAYLQVQASADGFDPSEQAAYEAFEAARVRASQELAASAETITKTRESVAYALKADREATAAFEAYLSALRQVSVINDLIADANAKNKTDFAEIELYDVLYTDADISGDAPLLAPAYKELKDLQAEVDADFEWLGEFAIDNNEDNYVIRTHIPAVEALKAAIDSLVDTVEPLRADAIAKNIEAQKSDVLVPQLFLERATAQRDTLRVVEAIFSTSARYVELYENVENVNVENKTLRQHYSSLIPNLFIAAVGNINELNNADQAARELFLDWDTDLTTNDEDEAYYQAKLDFAIETYAKILINGEVWQEPLAYVQNLDAGARQEAADREAERAADAAYRAEQLRIAQEAADAQKALAEALANAGNNDNGGDNSSDDKGTGSSDIGTWGPFAAIAAIIAAIAAIFPFLSGIVKF

SEQ ID NO: 12 - DNA, 318 bp, Corynebacterium glutamicum
  source 1..318: mol_type = genomic DNA
atgtccctcggaccatgggaaattggaatcattgtcctgctgatcatcgtgctgttcggcgcgaagaagctgcctgatgcagctcgttccatcggccgttccatgcgcatcttcaagtctgaagtcaaagaaatgaacaaggacggcgataccccagaacaacagcagcagcctcagcagcagattgcgcccaaccagatcgaggctcctcagccaaactttgagcagcactaccagggacagcaggttcagcagcctcagaaccctcagacccctgactaccgtcagaactacgaggatccaaaccgcacctcttaa

SEQ ID NO: 13 - protein, 105 aa, Corynebacterium glutamicum
MSLGPWEIGIIVLLIIVLFGAKKLPDAARSIGRSMRIFKSEVKEMNKDGDTPEQQQQPQQQIAPNQIEAPQPNFEQHYQGQQVQQPQNPQTPDYRQNYEDPNRTS

SEQ ID NO: 14 - DNA, 471 bp, Corynebacterium glutamicum
  source 1..471: mol_type = genomic DNA
atgttttctagcgtgggttggggagagatcttcctcttagtcgttgtgggccttgttgtcatcggcccggaacggttgcctcgtttgatccaggacgcacgcgctgcgctgctcgctgcacgtaccgctatcgacaatgcaaagcagtcgttggacagtgattttggttcggaatttgatgaaatccgaaagccactaacccaggttgcacagtacagccggatgagccccaagacggccatcactaaggcgttatttgataatgattcctcgttcctggatgactttgatccaaagaagatcatggccgaaggaacagaaggcgaagctcagcgcaacaagcaggcagctgacaacaatgcgaatgtggtggaacgtccagctgatggttccaccgcacgcccaacgcaaaacgatccaaaagacggcccgaattactcaggtggcgtctcttggaccgatattatttag

SEQ ID NO: 15 - protein, 156 aa, Corynebacterium glutamicum
MFSSVGWGEIFLLVVVGLVVIGPERLPRLIQDARAALLAARTAIDNAKQSLDSDFGSEFDEIRKPLTQVAQYSRMSPKTAITKALFDNDSSFLDDFDPKKIMAEGTEGEAQRNKQAADNNANVVERPADGSTARPTQNDPKDGPNYSGGVSWTDII

SEQ ID NO: 16 - DNA, 945 bp, Corynebacterium glutamicum
  source 1..945: mol_type = genomic DNA
atgtccattgttgagcacatcaaagagtttcgacgccgacttcttatcgctctggcgggcatcctcgtgggcaccattatcggctttatttggtacgatttctcattttggcagatccccactttgggcgagctgctgagggatccgtactgttctctgcctgctgaatcccgctgggccatgagcgactcagaggaatgtcgactgctcgcaaccggcccgtttgatccattcatgcttcgccttaaagtagcggcgttggtgggtatggttcttggctcacccgtgtggctgagccagctgtggggctttatcaccccaggtttgatgaagaatgagcgccgttacaccgcaatcttcgtcacgattgctgttgtgctgtttgtcggcggtgctgttcttgcgtacttcgtcgttgcatatggtttggagttcctccttaccattggtggagacacccaggcagcggccctgactggtgataagtacttcggattcttgctcgcgttgttggcgattttcggcgtgagcttcgaagttccactggtgatcggcatgctcaacattgtgggtatcttgccttacgatgccattaaagataagcgacgcatgatcatcatgattttgttcgtgttcgctgctttcatgacacccggccaggatcctttcaccatgttggtgttggcgctttcactcaccgttctggtagagcttgccctgcagttctgtcgtttcaacgacaaacgccgggacaagaagcgcccagaatggcttgatggcgatgacctctctgcatcaccactggatacttctgctggtggagaagatgctccaagcccagtcgaaaccccagaggcggtggagccttcgcggatgctgaacccaagtggggaggcgtcgataagctataaacccgggcgcgccgacttcggtgacgtgctctag

SEQ ID NO: 17 - protein, 314 aa, Corynebacterium glutamicum
MSIVEHIKEFRRRLLIALAGILVGTIIGFIWYDFSFWQIPTLGELLRDPYCSLPAESRWAMSDSEECRLLATGPFDPFMLRLKVAALVGMVLGSPVWLSQLWGFITPGLMKNERRYTAIFVTIAVVLFVGGAVLAYFVVAYGLEFLLTIGGDTQAAALTGDKYFGFLLALLAIFGVSFEVPLVIGMLNIVGILPYDAIKDKRRMIIMILFVFAAFMTPGQDPFTMLVLALSLTVLVELALQFCRFNDKRRDKKRPEWLDGDDLSASPLDTSAGGEDAPSPVETPEAVEPSRMLNPSGEASISYKPGRADFGDVL

SEQ ID NO: 18 - protein, 39 aa, Escherichia coli
MNNNDLFQASRRRFLAQLGGLTVAGMLGPSLLTPRRATA

SEQ ID NO: 19 - protein, 27 aa, Escherichia coli
MSLSRRQFIQASGIALCAGAVPLKASA

SEQ ID NO: 20 - protein, 48 aa, Bacillus subtilis
MAYDSRFDEWVQKLKEESFQNNTFDRRKFIQGAGKIAGLSLGLTIAQS

SEQ ID NO: 21 - protein, 34 aa, Bacillus subtilis
MKFVKRRTTALVTTLMLSVTSLFALQPSAKAAEH

SEQ ID NO: 22 - protein, 30 aa, Arthrobacter globiformis
MMNLSRRTLLTTGSAATLAYALGMAGSAQA

SEQ ID NO: 23 - protein, 7 aa, synthetic construct
  REGION 1..7: note = Twin-Arginine Motif
  SITE 1: note = misc_feature - Xaa can be any naturally occurring amino acid
  SITE 4: note = misc_feature - Xaa can be any naturally occurring amino acid
XRRXFLK

SEQ ID NO: 24 - skipped

SEQ ID NO: 25 - protein, 43 aa, Corynebacterium glutamicum
MRDTAFRSIKAKAQAKRRSLWIAAGAVPTAIALTMSLAPMASA

SEQ ID NO: 26 - protein, 30 aa, Corynebacterium glutamicum
MFNNRIRTAALAGAIAISTAASGVAIPAFA

SEQ ID NO: 27 - protein, 25 aa, Corynebacterium stationis
MKRMKSLAAALTVAGAMLAAPVATA

SEQ ID NO: 28 - protein, 469 aa, Corynebacterium glutamicum
QETNPTFNINNGFNDADGSTIQPVEPVNHTEETLRDLTDSTGAYLEEFQYGNVEEIVEAYLQVQASADGFDPSEQAAYEAFEAARVRASQELAASAETITKTRESVAYALKADREATAAFEAYLSALRQVSVINDLIADANAKNKTDFAEIELYDVLYTDADISGDAPLLAPAYKELKDLQAEVDADFEWLGEFAIDNNEDNYVIRTHIPAVEALKAAIDSLVDTVEPLRADAIAKNIEAQKSDVLVPQLFLERATAQRDTLRVVEAIFSTSARYVELYENVENVNVENKTLRQHYSSLIPNLFIAAVGNINELNNADQAARELFLDWDTDLTTNDEDEAYYQAKLDFAIETYAKILINGEVWQEPLAYVQNLDAGARQEAADREAERAADAAYRAEQLRIAQEAADAQKALAEALANAGNNDNGGDNSSDDKGTGSSDIGTWGPFAAIAAIIAAIAAIFPFLSGIVKF

SEQ ID NO: 29-31 - skipped (3 entries)

SEQ ID NO: 32 - protein, 6 aa, Corynebacterium glutamicum
QETNPT

SEQ ID NO: 33 - protein, 6 aa, Corynebacterium glutamicum
QETGTY

SEQ ID NO: 34 - protein, 6 aa, Corynebacterium glutamicum
QETTVT

SEQ ID NO: 35 - protein, 6 aa, Corynebacterium glutamicum
QETPVT

SEQ ID NO: 36 - protein, 6 aa, Corynebacterium glutamicum
QETAVT

SEQ ID NO: 37 - protein, 4 aa, synthetic construct
  REGION 1..4: note = Factor Xa
IEGR

SEQ ID NO: 38 - protein, 6 aa, synthetic construct
  REGION 1..6: note = ProTEV
ENLYFQ

SEQ ID NO: 39 - DNA, 987 bp, Corynebacterium glutamicum
  source 1..987: mol_type = genomic DNA
atgaattccccgcagaacgtttccaccaagaaggtcaccgtcaccggcgcagctggtcaaatctcttattcactgttgtggcgcatcgccaacggtgaagtattcggcaccgacacccctgtagaactgaaacttctggagatccctcaggctcttggcggggcagagggcgtggctatggaacttctggattctgccttccccctcctgcgaaacatcaccatcaccgcggatgccaatgaggcattcgacggcgctaatgcggcgtttttggtcggtgcgaagcctcgcggaaaaggcgaagagcgcgcagatctgctggctaacaacggcaagattttcggacctcaaggtaaagctatcaatgacaacgccgcagatgacattcgtgtcctagttgttggaaacccagcgaacaccaacgcgttgattgcttcagctgcggccccagatgttccagcatcccgcttcaacgcaatgatgcgccttgatcacaaccgtgcgatctcccagctggccaccaagcttggccgtggatctgcggaatttaacaacattgtggtctggggaaatcactccgcaacccagttcccagacatcacctacgcaaccgttggtggagaaaaggtcactgacctggttgatcacgattggtatgtggaggagttcattcctcgcgtggctaaccgtggtgctgaaatcattgaggtccgtggaaagtcttctgcagcttctgcagcatcctctgcgattgatcacatgcgcgattgggtacagggcaccgaggcgtggtcctctgcggcaattccttccaccggtggatacggcattcctgagggcatttttgtcggtctgccaaccgtatcccgcaacggtgagtgggaaatcgttgaaggcctggagatttccgatttccagcgtgcccgcatcgacgcgaatgctcaggaattgcaggccgagcgcgaggcagtgcgcgacttgctctaa

SEQ ID NO: 40 - protein, 328 aa, Corynebacterium glutamicum
MNSPQNVSTKKVTVTGAAGQISYSLLWRIANGEVFGTDTPVELKLLEIPQALGGAEGVAMELLDSAFPLLRNITITADANEAFDGANAAFLVGAKPRGKGEERADLLANNGKIFGPQGKAINDNAADDIRVLVVGNPANTNALIASAAAPDVPASRFNAMMRLDHNRAISQLATKLGRGSAEFNNIVVWGNHSATQFPDITYATVGGEKVTDLVDHDWYVEEFIPRVANRGAEIIEVRGKSSAASAASSAIDHMRDWVQGTEAWSSAAIPSTGGYGIPEGIFVGLPTVSRNGEWEIVEGLEISDFQRARIDANAQELQAEREAVRDLL

SEQ ID NO: 41 - DNA, 33 bp, synthetic construct
  misc_feature 1..33: note = primer
  source 1..33: mol_type = other DNA
tcgagctcggtaccccttcctctggtttccacc

SEQ ID NO: 42 - DNA, 35 bp, synthetic construct
  misc_feature 1..35: note = primer
  source 1..35: mol_type = other DNA
attgaggattgtttatctttaacgcatgacttcgc

SEQ ID NO: 43 - DNA, 21 bp, synthetic construct
  misc_feature 1..21: note = primer
  source 1..21: mol_type = other DNA
taaacaatcctcaatccttgt

SEQ ID NO: 44 - DNA, 33 bp, synthetic construct
  misc_feature 1..33: note = primer
  source 1..33: mol_type = other DNA
ctctagaggatcccccaacaaccaggtagctgg

SEQ ID NO: 45 - DNA, 33 bp, synthetic construct
  misc_feature 1..33: note = primer
  source 1..33: mol_type = other DNA
tcgagctcggtacccgtgttccgtgagcacgat

SEQ ID NO: 46 - DNA, 40 bp, synthetic construct
  misc_feature 1..40: note = primer
  source 1..40: mol_type = other DNA
gcccgcatcgacgcgtagtagaatgctcaggaattgcagg

SEQ ID NO: 47 - DNA, 18 bp, synthetic construct
  misc_feature 1..18: note = primer
  source 1..18: mol_type = other DNA
cgcgtcgatgcgggcacg

SEQ ID NO: 48 - DNA, 34 bp, synthetic construct
  misc_feature 1..34: note = primer
  source 1..34: mol_type = other DNA
ctctagaggatccccggctgttctcttttaagcg